European Patent Specification EP 4 416 301 B1, published June 11, 2025. Title: METHOD FOR THE DETERMINATION OF HYDROLYTIC ACTIVITY. Applicant: F. Hoffmann-La Roche AG. Application EP. The sequence listing filed with the application follows.

SEQUENCE LISTING (46 sequences)

SEQ ID NO: 1-16 - skipped (16 entries)

SEQ ID NO: 17 - DNA, 12 bp, synthetic construct
  misc_feature 1..12: note = tag-17
  source 1..12: mol_type = other DNA
caacacaccaac

SEQ ID NO: 18 - DNA, 10 bp, synthetic construct
  misc_feature 1..10: note = tag-18
  source 1..10: mol_type = other DNA
acacaccaac

SEQ ID NO: 19-22 - skipped (4 entries)

SEQ ID NO: 23 - DNA, 12 bp, synthetic construct
  misc_feature 1..12: note = tag-23
  source 1..12: mol_type = other DNA
gttggtgtgttg

SEQ ID NO: 24-30 - skipped (7 entries)

SEQ ID NO: 31 - DNA, 15 bp, synthetic construct
  misc_feature 1..15: note = tag-31
  source 1..15: mol_type = other DNA
gttggtgtgttggtg

SEQ ID NO: 32 - DNA, 15 bp, synthetic construct
  misc_feature 1..15: note = tag-32
  source 1..15: mol_type = other DNA
caccaacacaccaac

SEQ ID NO: 33-46 - skipped (14 entries)